European Patent Application EP 4 606 381 A1, published August 27, 2025. Title: 治疗或预防巨噬细胞介导的疾病的药物及其应用. Applicant: 安徽楚沅生物科技有限公司. Application CN. The sequence listing filed with the application follows.

SEQUENCE LISTING (14 sequences)

SEQ ID NO: 1 - DNA, 22 bp, synthetic construct
  source 1..22: mol_type = other DNA
gagggaagcgagagattatgga

SEQ ID NO: 2 - DNA, 21 bp, synthetic construct
  source 1..21: mol_type = other DNA
gcctgatgccaggttaaagca

SEQ ID NO: 3 - DNA, 20 bp, synthetic construct
  source 1..20: mol_type = other DNA
ttgggtggatgctcacactg

SEQ ID NO: 4 - DNA, 21 bp, synthetic construct
  source 1..21: mol_type = other DNA
gtacacgatgtctttggcaga

SEQ ID NO: 5 - DNA, 21 bp, synthetic construct
  source 1..21: mol_type = other DNA
acatcgacccgtccacagtat

SEQ ID NO: 6 - DNA, 20 bp, synthetic construct
  source 1..20: mol_type = other DNA
cagaggggtaggcttgtctc

SEQ ID NO: 7 - DNA, 20 bp, synthetic construct
  source 1..20: mol_type = other DNA
ctgaacttcggggtgatcgg

SEQ ID NO: 8 - DNA, 23 bp, synthetic construct
  source 1..23: mol_type = other DNA
ggcttgtcactcgaattttgaga

SEQ ID NO: 9 - DNA, 20 bp, synthetic construct
  source 1..20: mol_type = other DNA
ccaagaggtgagtgcttccc

SEQ ID NO: 10 - DNA, 22 bp, synthetic construct
  source 1..22: mol_type = other DNA
ctgttgttcagactctctccct

SEQ ID NO: 11 - DNA, 22 bp, synthetic construct
  source 1..22: mol_type = other DNA
gaaatgccaccttttgacagtg

SEQ ID NO: 12 - DNA, 21 bp, synthetic construct
  source 1..21: mol_type = other DNA
tggatgctctcatcaggacag

SEQ ID NO: 13 - DNA, 20 bp, synthetic construct
  source 1..20: mol_type = other DNA
ccagtatgactccactcacg

SEQ ID NO: 14 - DNA, 20 bp, synthetic construct
  source 1..20: mol_type = other DNA
gactccacgacatactcagc